European Patent Application EP 4 137 502 A1, published February 22, 2023. Title: VIPR2 Antagonist Peptide. Applicant: ICHIMARU PHARCOS Co., Ltd. The sequence listing filed with the application follows.

SEQUENCE LISTING (11 sequences)

SEQ ID NO: 1 - protein, 13 aa, Artificial Sequence
  VIPR2 antagonistic bicyclic peptide 1
  MOD_RES (1)..(1): 3-mercaptopropanoic acid (Mpa)
  DISULFID (1)..(10): S-S(1-10)
  MISC_FEATURE (7)..(11): Cyclization by amide linkage (7-11)
  MOD_RES (13)..(13): AMIDATION
XPPYLPKYLCDLI

SEQ ID NO: 2 - protein, 11 aa, Artificial Sequence
  VIPR2 antagonistic bicyclic peptide 2
  MOD_RES (1)..(1): 3-mercaptopropanoic acid (Mpa)
  THIOETH (1)..(8): Cyclization (1-8) by the reaction with 1,4-diiodobutane (DIBut)
  MOD_RES (2)..(2): N-methyl tyrosine (NmeTyr)
  MISC_FEATURE (5)..(9): Cyclization by amide linkage (5-9)
  MOD_RES (11)..(11): AMIDATION
XYLPKYLCDLI

SEQ ID NO: 3 - protein, 11 aa, Artificial Sequence
  VIPR2 antagonistic bicyclic peptide 3
  MOD_RES (1)..(1): 3-mercaptopropanoic acid (Mpa)
  THIOETH (1)..(8): Cyclization (1-8) by the reaction with 1,5-diiodopentane (DIPen)
  MOD_RES (2)..(2): N-methyl tyrosine (NmeTyr)
  MISC_FEATURE (5)..(9): Cyclization by amide linkage (5-9)
  MOD_RES (11)..(11): AMIDATION
XYLPKYLCDLI

SEQ ID NO: 4 - protein, 11 aa, Artificial Sequence
  VIPR2 antagonistic bicyclic peptide 4
  MOD_RES (1)..(1): 3-mercaptopropanoic acid (Mpa)
  THIOETH (1)..(8): Cyclization (1-8) by the reaction with 1,6-diiodohexane (DIHex)
  MOD_RES (2)..(2): N-methyl tyrosine (NmeTyr)
  MISC_FEATURE (5)..(9): Cyclization by amide linkage (5-9)
  MOD_RES (11)..(11): AMIDATION
XYLPKYLCDLI

SEQ ID NO: 5 - protein, 11 aa, Artificial Sequence
  VIPR2 antagonistic bicyclic peptide 5
  MOD_RES (1)..(1): 3-mercaptopropanoic acid (Mpa)
  THIOETH (1)..(8): Cyclization (1-8) by the reaction with 1,2-bis(bromomethyl)benzene (DBoXy (1-8)
  MOD_RES (2)..(2): N-methyl tyrosine (NmeTyr)
  MISC_FEATURE (5)..(9): Cyclization by amide linkage (5--9)
  MOD_RES (11)..(11): AMIDATION
XYLPKYLCDLI

SEQ ID NO: 6 - protein, 11 aa, Artificial Sequence
  VIPR2 antagonistic bicyclic peptide 6
  MOD_RES (1)..(1): 3-mercaptopropanoic acid (Mpa)
  THIOETH (1)..(8): Cyclization (1-8) by the reaction with 1,3-bis(bromomethyl)benzene (DBmXy )
  MOD_RES (2)..(2): N-methyl tyrosine (NmeTyr)
  MISC_FEATURE (5)..(9): Cyclization by amide linkage (5-9)
  MOD_RES (11)..(11): AMIDATION
XYLPKYLCDLI

SEQ ID NO: 7 - protein, 11 aa, Artificial Sequence
  VIPR2 antagonistic bicyclic peptide 7
  MOD_RES (1)..(1): 3-mercaptopropanoic acid (Mpa)
  THIOETH (1)..(8): Cyclization (1-8) by the reaction with 1,4-bis(bromomethyl)benzene (DBpXy)
  MOD_RES (2)..(2): N-methyl tyrosine (NmeTyr)
  MISC_FEATURE (5)..(9): Cyclization by amide linkage (5-9)
  MOD_RES (11)..(11): AMIDATION
XYLPKYLCDLI

SEQ ID NO: 8 - protein, 11 aa, Artificial Sequence
  VIPR2 antagonistic bicyclic peptide 8
  MOD_RES (1)..(1): 3-mercaptopropanoic acid (Mpa)
  MISC_FEATURE (1)..(5): trifurcate linkage by TBMB (1-5-8)
  MOD_RES (2)..(2): N-methyl tyrosine (NmeTyr)
  MOD_RES (4)..(4): METHYLATION, (MeGly)
  MISC_FEATURE (5)..(8): trifurcate linkage by TBMB (1-5-8)
  MOD_RES (11)..(11): AMIDATION
XYLGCYLCSLI

SEQ ID NO: 9 - protein, 11 aa, Artificial Sequence
  VIPR2 antagonistic bicyclic peptide 9
  MOD_RES (1)..(1): 3-mercaptopropanoic acid (Mpa)
  MISC_FEATURE (1)..(5): trifurcate linkage by TBMB (1-5-8)
  MOD_RES (2)..(2): N-methyl tyrosine (NmeTyr)
  MOD_RES (4)..(4): METHYLATION, (MeGly)
  MISC_FEATURE (5)..(8): trifurcate linkage by TBMB (1-5-8)
  MOD_RES (9)..(9): (S)-2,3-Diaminopropanoic acid (Dap)
  MOD_RES (11)..(11): AMIDATION
XYLGCYLCXLI

SEQ ID NO: 10 - protein, 13 aa, Artificial Sequence
  VIPR2 antagonistic bicyclic peptide 10
  MOD_RES (1)..(1): ACETYLATION
  DISULFID (1)..(10): S-S(1-10)
  MISC_FEATURE (7)..(11): Cyclization by amide linkage (7-11)
  MOD_RES (13)..(13): AMIDATION
CPPYLPKYLCDLI

SEQ ID NO: 11 - protein, 16 aa, Artificial Sequence
  cyclic peptide VIpep-3
  MOD_RES (1)..(1): ACETYLATION
  DISULFID (1)..(10)
CPPYLPRRLCTLLLRS